European Patent Specification EP 3 234 151 B1, published August 13, 2025. Title: FUNGAL GENOME MODIFICATION SYSTEMS AND METHODS OF USE. Applicant: Danisco US Inc Ward, Michael Chan, Jimmy Bower, Benjamin S Kim, Steven S Madrid, Susan M Ge, Jing Gu, Xiaogang Song, Danfeng Song, Mingmin. The sequence listing filed with the application follows.

SEQUENCE LISTING (92 sequences)

SEQ ID NO: 1 - protein, 1368 aa, Streptococcus pyogenes [sequence omitted]

SEQ ID NO: 2 - protein, 1388 aa, Streptococcus thermophilus
MTKPYSIGLDIGTNSVGWAVTTDNYKVPSKKMKVLGNTSKKYIKKNLLGVLLFDSGITAEGRRLKRTARRRYTRRRNRILYLQEIFSTEMATLDDAFFQRLDDSFLVPDDKRDSKYPIFGNLVEEKAYHDEFPTIYHLRKYLADSTKKADLRLVYLALAHMIKYRGHFLIEGEFNSKNNDIQKNFQDFLDTYNAIFESDLSLENSKQLEEIVKDKISKLEKKDRILKLFPGEKNSGIFSEFLKLIVGNQADFRKCFNLDEKASLHFSKESYDEDLETLLGYIGDDYSDVFLKAKKLYDAILLSGFLTVTDNETEAPLSSAMIKRYNEHKEDLALLKEYIRNISLKTYNEVFKDDTKNGYAGYIDGKTNQEDFYVYLKKLLAEFEGADYFLEKIDREDFLRKQRTFDNGSIPYQIHLQEMRAILDKQAKFYPFLAKNKERIEKILTFRIPYYVGPLARGNSDFAWSIRKRNEKITPWNFEDVIDKESSAEAFINRMTSFDLYLPEEKVLPKHSLLYETFNVYNELTKVRFIAESMRDYQFLDSKQKKDIVRLYFKDKRKVTDKDIIEYLHAIYGYDGIELKGIEKQFNSSLSTYHDLLNIINDKEFLDDSSNEAIIEEIIHTLTIFEDREMIKQRLSKFENIFDKSVLKKLSRRHYTGWGKLSAKLINGIRDEKSGNTILDYLIDDGISNRNFMQLIHDDALSFKKKIQKAQIIGDEDKGNIKEVVKSLPGSPAIKKGILQSIKIVDELVKVMGGRKPESIVVEMARENQYTNQGKSNSQQRLKRLEKSLKELGSKILKENIPAKLSKIDNNALQNDRLYLYYLQNGKDMYTGDDLDIDRLSNYDIDHIIPQAFLKDNSIDNKVLVSSASNRGKSDDVPSLEVVKKRKTFWYQLLKSKLISQRKFDNLTKAERGGLSPEDKAGFIQRQLVETRQITKHVARLLDEKFNNKKDENNRAVRTVKIITLKSTLVSQFRKDFELYKVREINDFHHAHDAYLNAVVASALLKKYPKLEPEFVYGDYPKYNSFRERKSATEKVYFYSNIMNIFKKSISLADGRVIERPLIEVNEETGESVWNKESDLATVRRVLSYPQVNVVKKVEEQNHGLDRGKPKGLFNANLSSKPKPNSNENLVGAKEYLDPKKYGGYAGISNSFTVLVKGTIEKGAKKKITNVLEFQGISILDRINYRKDKLNFLLEKGYKDIELIIELPKYSLFELSDGSRRMLASILSTNNKRGEIHKGNQIFLSQKFVKLLYHAKRISNTINENHRKYVENHKKEFEELFYYILEFNENYVGAKKNGKLLNSAFQSWQNHSIDELCSSFIGPTGSERKGLFELTSRGSAADFEFLGVKIPRYRDYTPSSLLKDATLIHQSVTGLYETRIDLAKLGEG

SEQ ID NO: 3 - protein, 1345 aa, Streptococcus mutans
MKKPYSIGLDIGTNSVGWAVVTDDYKVPAKKMKVLGNTDKSHIEKNLLGALLFDSGNTAEDRRLKRTARRRYTRRRNRILYLQEIFSEEMGKVDDSFFHRLEDSFLVTEDKRGERHPIFGNLEEEVKYHENFPTIYHLRQYLADNPEKVDLRLVYLALAHIIKFRGHFLIEGKFDTRNNDVQRLFQEFLAVYDNTFENSSLQEQNVQVEEILTDKISKSAKKDRVLKLFPNEKSNGRFAEFLKLIVGNQADFKKHFELEEKAPLQFSKDTYEEELEVLLAQIGDNYAELFLSAKKLYDSILLSGILTVTDVGTKAPLSASMIQRYNEHQMDLAQLKQFIRQKLSDKYNEVFSDVSKDGYAGYIDGKTNQEAFYKYLKGLLNKIEGSGYFLDKIEREDFLRKQRTFDNGSIPHQIHLQEMRAIIRRQAEFYPFLADNQDRIEKLLTFRIPYYVGPLARGKSDFAWLSRKSADKITPWNFDEIVDKESSAEAFINRMTNYDLYLPNQKVLPKHSLLYEKFTVYNELTKVKYKTEQGKTAFFDANMKQEIFDGVFKVYRKVTKDKLMDFLEKEFDEFRIVDLTGLDKENKVFNASYGTYHDLCKILDKDFLDNSKNEKILEDIVLTLTLFEDREMIRKRLENYSDLLTKEQVKKLERRHYTGWGRLSAELIHGIRNKESRKTILDYLIDDGNSNRNFMQLINDDALSFKEEIAKAQVIGETDNLNQVVSDIAGSPAIKKGILQSLKIVDELVKIMGHQPENIVVEMARENQFTNQGRRNSQQRLKGLTDSIKEFGSQILKEHPVENSQLQNDRLFLYYLQNGRDMYTGEELDIDYLSQYDIDHIIPQAFIKDNSIDNRVLTSSKENRGKSDDVPSKDVVRKMKSYWSKLLSAKLITQRKFDNLTKAERGGLTDDDKAGFIKRQLVETRQITKHVARILDERFNTETDENNKKIRQVKIVTLKSNLVSNFRKEFELYKVREINDYHHAHDAYLNAVIGKALLGVYPQLEPEFVYGDYPHFHGHKENKATAKKFFYSNIMNFFKKDDVRTDKNGEIIWKKDEHISNIKKVLSYPQVNIVKKVEEQTGGFSKESILPKGNSDKLIPRKTKKFYWDTKKYGGFDSPIVAYSILVIADIEKGKSKKLKTVKALVGVTIMEKMTFERDPVAFLERKGYRNVQEENIIKLPKYSLFKLENGRKRLLASARELQKGNEIVLPNHLGTLLYHAKNIHKVDEPKHLDYVDKHKDEFKELLDVVSNFSKKYTLAEGNLEKIKELYAQNNGEDLKELASSFINLLTFTAIGAPATFKFFDKNIDRKRYTSTTEILNATLIHQSITGLYETRIDLNKLGGD

SEQ ID NO: 4 - protein, 984 aa, Campylobacter jejuni
MARILAFDIGISSIGWAFSENDELKDCGVRIFTKVENPKTGESLALPRRLARSARKRLARRKARLNHLKHLIANEFKLNYEDYQSFDESLAKAYKGSLISPYELRFRALNELLSKQDFARVILHIAKRRGYDDIKNSDDKEKGAILKAIKQNEEKLANYQSVGEYLYKEYFQKFKENSKEFTNVRNKKESYERCIAQSFLKDELKLIFKKQREFGFSFSKKFEEEVLSVAFYKRALKDFSHLVGNCSFFTDEKRAPKNSPLAFMFVALTRIINLLNNLKNTEGILYTKDDLNALLNEVLKNGTLTYKQTKKLLGLSDDYEFKGEKGTYFIEFKKYKEFIKALGEHNLSQDDLNEIAKDITLIKDEIKLKKALAKYDLNQNQIDSLSKLEFKDHLNISFKALKLVTPLMLEGKKYDEACNELNLKVAINEDKKDFLPAFNETYYKDEVTNPVVLRAIKEYRKVLNALLKKYGKVHKINIELAREVGKNHSQRAKIEKEQNENYKAKKDAELECEKLGLKINSKNILKLRLFKEQKEFCAYSGEKIKISDLQDEKMLEIDHIYPYSRSFDDSYMNKVLVFTKQNQEKLNQTPFEAFGNDSAKWQKIEVLAKNLPTKKQKRILDKNYKDKEQKNFKDRNLNDTRYIARLVLNYTKDYLDFLPLSDDENTKLNDTQKGSKVHVEAKSGMLTSALRHTWGFSAKDRNNHLHHAIDAVIIAYANNSIVKAFSDFKKEQESNSAELYAKKISELDYKNKRKFFEPFSGFRQKVLDKIDEIFVSKPERKKPSGALHEETFRKEEEFYQSYGGKEGVLKALELGKIRKVNGKIVKNGDMFRVDIFKHKKTNKFYAVPIYTMDFALKVLPNKAVARSKKGEIKDWILMDENYEFCFSLYKDSLILIQTKDMQEPEFVYYNAFTSSTVSLIVSKHDNKFETLSKNQKILFKNANEKEVIAKSIGIQNLKVFEKYIVSALGEVTKAEFRQREDFKK

SEQ ID NO: 5 - protein, 1082 aa, Neisseria meningitides
MAAFKPNSINYILGLDIGIASVGWAMVEIDEEENPIRLIDLGVRVFERAEVPKTGDSLAMARRLARSVRRLTRRRAHRLLRTRRLLKREGVLQAANFDENGLIKSLPNTPWQLRAAALDRKLTPLEWSAVLLHLIKHRGYLSQRKNEGETADKELGALLKGVAGNAHALQTGDFRTPAELALNKFEKESGHIRNQRSDYSHTFSRKDLQAELILLFEKQKEFGNPHVSGGLKEGIETLLMTQRPALSGDAVQKMLGHCTFEPAEPKAAKNTYTAERFIWLTKLNNLRILEQGSERPLTDTERATLMDEPYRKSKLTYAQARKLLGLEDTAFFKGLRYGKDNAEASTLMEMKAYHAISRALEKEGLKDKKSPLNLSPELQDEIGTAFSLFKTDEDITGRLKDRIQPEILEALLKHISFDKFVQISLKALRRIVPLMEQGKRYDEACAEIYGDHYGKKNTEEKIYLPPIPADEIRNPVVLRALSQARKVINGVVRRYGSPARIHIETAREVGKSFKDRKEIEKRQEENRKDREKAAAKFREYFPNFVGEPKSKDILKLRLYEQQHGKCLYSGKEINLGRLNEKGYVEIDHALPFSRTWDDSFNNKVLVLGSENQNKGNQTPYEYFNGKDNSREWQEFKARVETSRFPRSKKQRILLQKFDEDGFKERNLNDTRYVNRFLCQFVADRMRLTGKGKKRVFASNGQITNLLRGFWGLRKVRAENDRHHALDAVVVACSTVAMQQKITRFVRYKEMNAFDGKTIDKETGEVLHQKTHFPQPWEFFAQEVMIRVFGKPDGKPEFEEADTLEKLRTLLAEKLSSRPEAVHEYVTPLFVSRAPNRKMSGQGHMETVKSAKRLDEGVSVLRVPLTQLKLKDLEKMVNREREPKLYEALKARLEAHKDDPAKAFAEPFYKYDKAGNRTQQVKAVRVEQVQKTGVWVRNHNGIADNATMVRVDVFEKGDKYYLVPIYSWQVAKGILPDRAVVQGKDEEDWQLIDDSFNFKFSLHPNDLVEVITKKARMFGYFASCHRGTGNINIRIHDLDHKIGKNGILEGIGVKTALSFQKYQIDELGKEIRPCRLKKRPPVR

SEQ ID NO: 6 - protein, 1629 aa, Francisella tularensis
MNFKILPIAIDLGVKNTGVFSAFYQKGTSLERLDNKNGKVYELSKDSYTLLMNNRTARRHQRRGIDRKQLVKRLFKLIWTEQLNLEWDKDTQQAISFLFNRRGFSFITDGYSPEYLNIVPEQVKAILMDIFDDYNGEDDLDSYLKLATEQESKISEIYNKLMQKILEFKLMKLCTDIKDDKVSTKTLKEITSYEFELLADYLANYSESLKTQKFSYTDKQGNLKELSYYHHDKYNIQEFLKRHATINDRILDTLLTDDLDIWNFNFEKFDFDKNEEKLQNQEDKDHIQAHLHHFVFAVNKIKSEMASGGRHRSQYFQEITNVLDENNHQEGYLKNFCENLHNKKYSNLSVKNLVNLIGNLSNLELKPLRKYFNDKIHAKADHWDEQKFTETYCHWILGEWRVGVKDQDKKDGAKYSYKDLCNELKQKVTKAGLVDFLLELDPCRTIPPYLDNNNRKPPKCQSLILNPKFLDNQYPNWQQYLQELKKLQSIQNYLDSFETDLKVLKSSKDQPYFVEYKSSNQQIASGQRDYKDLDARILQFIFDRVKASDELLLNEIYFQAKKLKQKASSELEKLESSKKLDEVIANSQLSQILKSQHTNGIFEQGTFLHLVCKYYKQRQRARDSRLYIMPEYRYDKKLHKYNNTGRFDDDNQLLTYCNHKPRQKRYQLLNDLAGVLQVSPNFLKDKIGSDDDLFISKWLVEHIRGFKKACEDSLKIQKDNRGLLNHKINIARNTKGKCEKEIFNLICKIEGSEDKKGNYKHGLAYELGVLLFGEPNEASKPEFDRKIKKFNSIYSFAQIQQIAFAERKGNANTCAVCSADNAHRMQQIKITEPVEDNKDKIILSAKAQRLPAIPTRIVDGAVKKMATILAKNIVDDNWQNIKQVLSAKHQLHIPIITESNAFEFEPALADVKGKSLKDRRKKALERISPENIFKDKNNRIKEFAKGISAYSGANLTDGDFDGAKEELDHIIPRSHKKYGTLNDEANLICVTRGDNKNKGNRIFCLRDLADNYKLKQFETTDDLEIEKKIADTIWDANKKDFKFGNYRSFINLTPQEQKAFRHALFLADENPIKQAVIRAINNRNRTFVNGTQRYFAEVLANNIYLRAKKENLNTDKISFDYFGIPTIGNGRGIAEIRQLYEKVDSDIQAYAKGDKPQASYSHLIDAMLAFCIAADEHRNDGSIGLEIDKNYSLYPLDKNTGEVFTKDIFSQIKITDNEFSDKKLVRKKAIEGFNTHRQMTRDGIYAENYLPILIHKELNEVRKGYTWKNSEEIKIFKGKKYDIQQLNNLVYCLKFVDKPISIDIQISTLEELRNILTTNNIAATAEYYYINLKTQKLHEYYIENYNTALGYKKYSKEMEFLRSLAYRSERVKIKSIDDVKQVLDKDSNFIIGKITLPFKKEWQRLYREWQNTTIKDDYEFLKSFFNVKSITKLHKKVRKDFSLPISTNEGKFLVKRKTWDNNFIYQILNDSDSRADGTKPFIPAFDISKNEIVEAIIDSFTSKNIFWLPKNIELQKVDNKNIFAIDTSKWFEVETPSDLRDIGIATIQYKIDNNSRPKVRVKLDYVIDDDSKINYFMNHSLLKSRYPDKVLEILKQSTIIEFESSGFNKTIKEMLGMKLAGIYNETSNN

SEQ ID NO: 7 - protein, 1056 aa, Pasteurella multocida
MQTTNLSYILGLDLGIASVGWAVVEINENEDPIGLIDVGVRIFERAEVPKTGESLALSRRLARSTRRLIRRRAHRLLLAKRFLKREGILSTIDLEKGLPNQAWELRVAGLERRLSAIEWGAVLLHLIKHRGYLSKRKNESQTNNKELGALLSGVAQNHQLLQSDDYRTPAELALKKFAKEEGHIRNQRGAYTHTFNRLDLLAELNLLFAQQHQFGNPHCKEHIQQYMTELLMWQKPALSGEAILKMLGKCTHEKNEFKAAKHTYSAERFVWLTKLNNLRILEDGAERALNEEERQLLINHPYEKSKLTYAQVRKLLGLSEQAIFKHLRYSKENAESATFMELKAWHAIRKALENQGLKDTWQDLAKKPDLLDEIGTAFSLYKTDEDIQQYLTNKVPNSVINALLVSLNFDKFIELSLKSLRKILPLMEQGKRYDQACREIYGHHYGEANQKTSQLLPAIPAQEIRNPVVLRTLSQARKVINAIIRQYGSPARVHIETGRELGKSFKERREIQKQQEDNRTKRESAVQKFKELFSDFSSEPKSKDILKFRLYEQQHGKCLYSGKEINIHRLNEKGYVEIDHALPFSRTWDDSFNNKVLVLASENQNKGNQTPYEWLQGKINSERWKNFVALVLGSQCSAAKKQRLLTQVIDDNKFIDRNLNDTRYIARFLSNYIQENLLLVGKNKKNVFTPNGQITALLRSRWGLIKARENNNRHHALDAIVVACATPSMQQKITRFIRFKEVHPYKIENRYEMVDQESGEIISPHFPEPWAYFRQEVNIRVFDNHPDTVLKEMLPDRPQANHQFVQPLFVSRAPTRKMSGQGHMETIKSAKRLAEGISVLRIPLTQLKPNLLENMVNKEREPALYAGLKARLAEFNQDPAKAFATPFYKQGGQQVKAIRVEQVQKSGVLVRENNGVADNASIVRTDVFIKNNKFFLVPIYTWQVAKGILPNKAIVAHKNEDEWEEMDEGAKFKFSLFPNDLVELKTKKEYFFGYYIGLDRATGNISLKEHDGEISKGKDGVYRVGVKLALSFEKYQVDELGKNRQICRPQQRQPVR

SEQ ID NO: 8 - DNA, 4104 bp, Artificial sequence
  codon optimized gene
atggacaagaagtacagcatcggcctcgacatcggcaccaactcggtgggctgggccgtcatcacggacgaatataaggtcccgtcgaagaagttcaaggtcctcggcaatacagaccgccacagcatcaagaaaaacttgatcggcgccctcctgttcgatagcggcgagaccgcggaggcgaccaggctcaagaggaccgccaggagacggtacactaggcgcaagaacaggatctgctacctgcaggagatcttcagcaacgagatggcgaaggtggacgactccttcttccaccgcctggaggaatcattcctggtggaggaggacaagaagcatgagcggcacccaatcttcggcaacatcgtcgacgaggtggcctaccacgagaagtacccgacaatctaccacctccggaagaaactggtggacagcacagacaaggcggacctccggctcatctaccttgccctcgcgcatatgatcaagttccgcggccacttcctcatcgagggcgacctgaacccggacaactccgacgtggacaagctgttcatccagctcgtgcagacgtacaatcaactgttcgaggagaaccccataaacgctagcggcgtggacgccaaggccatcctctcggccaggctctcgaaatcaagaaggctggagaaccttatcgcgcagttgccaggcgaaaagaagaacggcctcttcggcaaccttattgcgctcagcctcggcctgacgccgaacttcaaatcaaacttcgacctcgcggaggacgccaagctccagctctcaaaggacacctacgacgacgacctcgacaacctcctggcccagataggagaccagtacgcggacctcttcctcgccgccaagaacctctccgacgctatcctgctcagcgacatccttcgggtcaacaccgaaattaccaaggcaccgctgtccgccagcatgattaaacgctacgacgagcaccatcaggacctcacgctgctcaaggcactcgtccgccagcagctccccgagaagtacaaggagatcttcttcgaccaatcaaaaaacggctacgcgggatatatcgacggcggtgccagccaggaagagttctacaagttcatcaaaccaatcctggagaagatggacggcaccgaggagttgctggtcaagctcaacagggaggacctcctcaggaagcagaggaccttcgacaacggctccatcccgcatcagatccacctgggcgaactgcatgccatcctgcggcgccaggaggacttctacccgttcctgaaggataaccgggagaagatcgagaagatcttgacgttccgcatcccatactacgtgggcccgctggctcgcggcaactcccggttcgcctggatgacccggaagtcggaggagaccatcacaccctggaactttgaggaggtggtcgataagggcgctagcgctcagagcttcatcgagcgcatgaccaacttcgataaaaacctgcccaatgaaaaagtcctccccaagcactcgctgctctacgagtacttcaccgtgtacaacgagctcaccaaggtcaaatacgtcaccgagggcatgcggaagccggcgttcctgagcggcgagcagaagaaggcgatagtggacctcctcttcaagaccaacaggaaggtgaccgtgaagcaattaaaagaggactacttcaagaaaatagagtgcttcgactccgtggagatctcgggcgtggaggatcggttcaacgcctcactcggcacgtatcacgacctcctcaagatcattaaagacaaggacttcctcgacaacgaggagaacgaggacatcctcgaggacatcgtcctcaccctgaccctgttcgaggaccgcgaaatgatcgaggagaggctgaagacctacgcgcacctgttcgacgacaaggtcatgaaacagctcaagaggcgccgctacactggttggggaaggctgtcccgcaagctcattaatggcatcagggacaagcagagcggcaagaccatcctggacttcctcaagtccgacgggttcgccaaccgcaacttcatgcagctcattcacgacgactcgctcacgttcaaggaagacatccagaaggcacaggtgagcgggcagggtgactccctccacgaacacatcgccaacctggccggctcgccggccattaaaaagggcatcctgcagacggtcaaggtcgtcgacgagctcgtgaaggtgatgggccggcacaagcccgaaaatatcgtcatagagatggccagggagaaccagaccacccaaaaagggcagaagaactcgcgcgagcggatgaaacggatcgaggagggcattaaagagctcgggtcccagatcctgaaggagcaccccgtggaaaatacccagctccagaatgaaaagctctacctctactacctgcagaacggccgcgacatgtacgtggaccaggagctggacattaatcggctatcggactacgacgtcgaccacatcgtgccgcagtcgttcctcaaggacgatagcatcgacaacaaggtgctcacccggtcggataaaaatcggggcaagagcgacaacgtgcccagcgaggaggtcgtgaagaagatgaaaaactactggcgccagctcctcaacgcgaaactgatcacccagcgcaagttcgacaacctgacgaaggcggaacgcggtggcttgagcgaactcgataaggcgggcttcataaaaaggcagctggtcgagacgcgccagatcacgaagcatgtcgcccagatcctggacagccgcatgaatactaagtacgatgaaaacgacaagctgatccgggaggtgaaggtgatcacgctgaagtccaagctcgtgtcggacttccgcaaggacttccagttctacaaggtccgcgagatcaacaactaccaccacgcccacgacgcctacctgaatgcggtggtcgggaccgccctgatcaagaagtacccgaagctggagtcggagttcgtgtacggcgactacaaggtctacgacgtgcgcaaaatgatcgccaagtccgagcaggagatcggcaaggccacggcaaaatacttcttctactcgaacatcatgaacttcttcaagaccgagatcaccctcgcgaacggcgagatccgcaagcgcccgctcatcgaaaccaacggcgagacgggcgagatcgtctgggataagggccgggatttcgcgacggtccgcaaggtgctctccatgccgcaagtcaatatcgtgaaaaagacggaggtccagacgggcgggttcagcaaggagtccatcctcccgaagcgcaactccgacaagctcatcgcgaggaagaaggattgggacccgaaaaaatatggcggcttcgacagcccgaccgtcgcatacagcgtcctcgtcgtggcgaaggtggagaagggcaagtcaaagaagctcaagtccgtgaaggagctgctcgggatcacgattatggagcggtcctccttcgagaagaacccgatcgacttcctagaggccaagggatataaggaggtcaagaaggacctgattattaaactgccgaagtactcgctcttcgagctggaaaacggccgcaagaggatgctcgcctccgcaggcgagttgcagaagggcaacgagctcgccctcccgagcaaatacgtcaatttcctgtacctcgctagccactatgaaaagctcaagggcagcccggaggacaacgagcagaagcagctcttcgtggagcagcacaagcattacctggacgagatcatcgagcagatcagcgagttctcgaagcgggtgatcctcgccgacgcgaacctggacaaggtgctgtcggcatataacaagcaccgcgacaaaccaatacgcgagcaggccgaaaatatcatccacctcttcaccctcaccaacctcggcgctccggcagccttcaagtacttcgacaccacgattgaccggaagcggtacacgagcacgaaggaggtgctcgatgcgacgctgatccaccagagcatcacagggctctatgaaacacgcatcgacctgagccagctgggcggagac

SEQ ID NO: 9 - DNA, 4155 bp, Artificial sequence
  codon optimized gene
atggcaccgaagaagaagcgcaaggtgatggacaagaagtacagcatcggcctcgacatcggcaccaactcggtgggctgggccgtcatcacggacgaatataaggtcccgtcgaagaagttcaaggtcctcggcaatacagaccgccacagcatcaagaaaaacttgatcggcgccctcctgttcgatagcggcgagaccgcggaggcgaccaggctcaagaggaccgccaggagacggtacactaggcgcaagaacaggatctgctacctgcaggagatcttcagcaacgagatggcgaaggtggacgactccttcttccaccgcctggaggaatcattcctggtggaggaggacaagaagcatgagcggcacccaatcttcggcaacatcgtcgacgaggtggcctaccacgagaagtacccgacaatctaccacctccggaagaaactggtggacagcacagacaaggcggacctccggctcatctaccttgccctcgcgcatatgatcaagttccgcggccacttcctcatcgagggcgacctgaacccggacaactccgacgtggacaagctgttcatccagctcgtgcagacgtacaatcaactgttcgaggagaaccccataaacgctagcggcgtggacgccaaggccatcctctcggccaggctctcgaaatcaagaaggctggagaaccttatcgcgcagttgccaggcgaaaagaagaacggcctcttcggcaaccttattgcgctcagcctcggcctgacgccgaacttcaaatcaaacttcgacctcgcggaggacgccaagctccagctctcaaaggacacctacgacgacgacctcgacaacctcctggcccagataggagaccagtacgcggacctcttcctcgccgccaagaacctctccgacgctatcctgctcagcgacatccttcgggtcaacaccgaaattaccaaggcaccgctgtccgccagcatgattaaacgctacgacgagcaccatcaggacctcacgctgctcaaggcactcgtccgccagcagctccccgagaagtacaaggagatcttcttcgaccaatcaaaaaacggctacgcgggatatatcgacggcggtgccagccaggaagagttctacaagttcatcaaaccaatcctggagaagatggacggcaccgaggagttgctggtcaagctcaacagggaggacctcctcaggaagcagaggaccttcgacaacggctccatcccgcatcagatccacctgggcgaactgcatgccatcctgcggcgccaggaggacttctacccgttcctgaaggataaccgggagaagatcgagaagatcttgacgttccgcatcccatactacgtgggcccgctggctcgcggcaactcccggttcgcctggatgacccggaagtcggaggagaccatcacaccctggaactttgaggaggtggtcgataagggcgctagcgctcagagcttcatcgagcgcatgaccaacttcgataaaaacctgcccaatgaaaaagtcctccccaagcactcgctgctctacgagtacttcaccgtgtacaacgagctcaccaaggtcaaatacgtcaccgagggcatgcggaagccggcgttcctgagcggcgagcagaagaaggcgatagtggacctcctcttcaagaccaacaggaaggtgaccgtgaagcaattaaaagaggactacttcaagaaaatagagtgcttcgactccgtggagatctcgggcgtggaggatcggttcaacgcctcactcggcacgtatcacgacctcctcaagatcattaaagacaaggacttcctcgacaacgaggagaacgaggacatcctcgaggacatcgtcctcaccctgaccctgttcgaggaccgcgaaatgatcgaggagaggctgaagacctacgcgcacctgttcgacgacaaggtcatgaaacagctcaagaggcgccgctacactggttggggaaggctgtcccgcaagctcattaatggcatcagggacaagcagagcggcaagaccatcctggacttcctcaagtccgacgggttcgccaaccgcaacttcatgcagctcattcacgacgactcgctcacgttcaaggaagacatccagaaggcacaggtgagcgggcagggtgactccctccacgaacacatcgccaacctggccggctcgccggccattaaaaagggcatcctgcagacggtcaaggtcgtcgacgagctcgtgaaggtgatgggccggcacaagcccgaaaatatcgtcatagagatggccagggagaaccagaccacccaaaaagggcagaagaactcgcgcgagcggatgaaacggatcgaggagggcattaaagagctcgggtcccagatcctgaaggagcaccccgtggaaaatacccagctccagaatgaaaagctctacctctactacctgcagaacggccgcgacatgtacgtggaccaggagctggacattaatcggctatcggactacgacgtcgaccacatcgtgccgcagtcgttcctcaaggacgatagcatcgacaacaaggtgctcacccggtcggataaaaatcggggcaagagcgacaacgtgcccagcgaggaggtcgtgaagaagatgaaaaactactggcgccagctcctcaacgcgaaactgatcacccagcgcaagttcgacaacctgacgaaggcggaacgcggtggcttgagcgaactcgataaggcgggcttcataaaaaggcagctggtcgagacgcgccagatcacgaagcatgtcgcccagatcctggacagccgcatgaatactaagtacgatgaaaacgacaagctgatccgggaggtgaaggtgatcacgctgaagtccaagctcgtgtcggacttccgcaaggacttccagttctacaaggtccgcgagatcaacaactaccaccacgcccacgacgcctacctgaatgcggtggtcgggaccgccctgatcaagaagtacccgaagctggagtcggagttcgtgtacggcgactacaaggtctacgacgtgcgcaaaatgatcgccaagtccgagcaggagatcggcaaggccacggcaaaatacttcttctactcgaacatcatgaacttcttcaagaccgagatcaccctcgcgaacggcgagatccgcaagcgcccgctcatcgaaaccaacggcgagacgggcgagatcgtctgggataagggccgggatttcgcgacggtccgcaaggtgctctccatgccgcaagtcaatatcgtgaaaaagacggaggtccagacgggcgggttcagcaaggagtccatcctcccgaagcgcaactccgacaagctcatcgcgaggaagaaggattgggacccgaaaaaatatggcggcttcgacagcccgaccgtcgcatacagcgtcctcgtcgtggcgaaggtggagaagggcaagtcaaagaagctcaagtccgtgaaggagctgctcgggatcacgattatggagcggtcctccttcgagaagaacccgatcgacttcctagaggccaagggatataaggaggtcaagaaggacctgattattaaactgccgaagtactcgctcttcgagctggaaaacggccgcaagaggatgctcgcctccgcaggcgagttgcagaagggcaacgagctcgccctcccgagcaaatacgtcaatttcctgtacctcgctagccactatgaaaagctcaagggcagcccggaggacaacgagcagaagcagctcttcgtggagcagcacaagcattacctggacgagatcatcgagcagatcagcgagttctcgaagcgggtgatcctcgccgacgcgaacctggacaaggtgctgtcggcatataacaagcaccgcgacaaaccaatacgcgagcaggccgaaaatatcatccacctcttcaccctcaccaacctcggcgctccggcagccttcaagtacttcgacaccacgattgaccggaagcggtacacgagcacgaaggaggtgctcgatgcgacgctgatccaccagagcatcacagggctctatgaaacacgcatcgacctgagccagctgggcggagacaagaagaagaagctcaagctctag

SEQ ID NO: 10 - protein, 1384 aa, Artificial sequence
  synthetic construct
MAPKKKRKVMDKKYSIGLDIGTNSVGWAVITDEYKVPSKKFKVLGNTDRHSIKKNLIGALLFDSGETAEATRLKRTARRRYTRRKNRICYLQEIFSNEMAKVDDSFFHRLEESFLVEEDKKHERHPIFGNIVDEVAYHEKYPTIYHLRKKLVDSTDKADLRLIYLALAHMIKFRGHFLIEGDLNPDNSDVDKLFIQLVQTYNQLFEENPINASGVDAKAILSARLSKSRRLENLIAQLPGEKKNGLFGNLIALSLGLTPNFKSNFDLAEDAKLQLSKDTYDDDLDNLLAQIGDQYADLFLAAKNLSDAILLSDILRVNTEITKAPLSASMIKRYDEHHQDLTLLKALVRQQLPEKYKEIFFDQSKNGYAGYIDGGASQEEFYKFIKPILEKMDGTEELLVKLNREDLLRKQRTFDNGSIPHQIHLGELHAILRRQEDFYPFLKDNREKIEKILTFRIPYYVGPLARGNSRFAWMTRKSEETITPWNFEEVVDKGASAQSFIERMTNFDKNLPNEKVLPKHSLLYEYFTVYNELTKVKYVTEGMRKPAFLSGEQKKAIVDLLFKTNRKVTVKQLKEDYFKKIECFDSVEISGVEDRFNASLGTYHDLLKIIKDKDFLDNEENEDILEDIVLTLTLFEDREMIEERLKTYAHLFDDKVMKQLKRRRYTGWGRLSRKLINGIRDKQSGKTILDFLKSDGFANRNFMQLIHDDSLTFKEDIQKAQVSGQGDSLHEHIANLAGSPAIKKGILQTVKVVDELVKVMGRHKPENIVIEMARENQTTQKGQKNSRERMKRIEEGIKELGSQILKEHPVENTQLQNEKLYLYYLQNGRDMYVDQELDINRLSDYDVDHIVPQSFLKDDSIDNKVLTRSDKNRGKSDNVPSEEVVKKMKNYWRQLLNAKLITQRKFDNLTKAERGGLSELDKAGFIKRQLVETRQITKHVAQILDSRMNTKYDENDKLIREVKVITLKSKLVSDFRKDFQFYKVREINNYHHAHDAYLNAVVGTALIKKYPKLESEFVYGDYKVYDVRKMIAKSEQEIGKATAKYFFYSNIMNFFKTEITLANGEIRKRPLIETNGETGEIVWDKGRDFATVRKVLSMPQVNIVKKTEVQTGGFSKESILPKRNSDKLIARKKDWDPKKYGGFDSPTVAYSVLVVAKVEKGKSKKLKSVKELLGITIMERSSFEKNPIDFLEAKGYKEVKKDLIIKLPKYSLFELENGRKRMLASAGELQKGNELALPSKYVNFLYLASHYEKLKGSPEDNEQKQLFVEQHKHYLDEIIEQISEFSKRVILADANLDKVLSAYNKHRDKPIREQAENIIHLFTLTNLGAPAAFKYFDTTIDRKRYTSTKEVLDATLIHQSITGLYETRIDLSQLGGDKKKKLKL

SEQ ID NO: 11 - DNA, 404 bp, Trichoderma reesei
aaaaaacactagtaagtacttacttatgtattattaactactttagctaacttctgcagtactacctaagaggctaggggtagttttatagcagacttatagctattatttttatttagtaaagtgcttttaaagtaaggtcttttttatagcactttttatttattataatatatattatataataattttaagcctggaatagtaaagaggcttatataataatttatagtaataaaagcttagcagctgtaatataattcctaaagaaacagcatgaaatggtattatgtaagagctatagtctaaaggcactctgctggataaaaatagtggctataagtctgctgcaaaactacccccaacctcgtaggtatataagtactgtttgatggtagtctatc

SEQ ID NO: 12 - DNA, 146 bp, Trichoderma reesei
aattcctaaagaaacagcatgaaatggtattatgtaagagctatagtctaaaggcactctgctggataaaaatagtggctataagtctgctgcaaaactacccccaacctcgtaggtatataagtactgtttgatggtagtctatc

SEQ ID NO: 13 - DNA, 138 bp, Artificial sequence
  synthetic construct
atgcaccatcatcatcatcattcttctggtctggtgccacgcggttctggtatgaaagaaaccgctgctgctaaattcgaacgccagcacatggacagcccagatctgggtaccgacgacgacgacaaggccatggcc

SEQ ID NO: 14 - DNA, 21 bp, SV40
ccaaaaaagaaacgcaaggtt

SEQ ID NO: 15 - DNA, 4104 bp, Artificial sequence
  synthetic construct
atggataaaaaatacagcattggtctggatatcggaaccaacagcgttgggtgggcagtaataacagatgaatacaaagtgccgtcaaaaaaatttaaggttctggggaatacagatcgccacagcataaaaaagaatctgattggggcattgctgtttgattcgggtgagacagctgaggccacgcgtctgaaacgtacagcaagaagacgttacacacgtcgtaaaaatcgtatttgctacttacaggaaattttttctaacgaaatggccaaggtagatgatagtttcttccatcgtctcgaagaatcttttctggttgaggaagataaaaaacacgaacgtcaccctatctttggcaatatcgtggatgaagtggcctatcatgaaaaataccctacgatttatcatcttcgcaagaagttggttgatagtacggacaaagcggatctgcgtttaatctatcttgcgttagcgcacatgatcaaatttcgtggtcatttcttaattgaaggtgatctgaatcctgataactctgatgtggacaaattgtttatacaattagtgcaaacctataatcagctgttcgaggaaaaccccattaatgcctctggagttgatgccaaagcgattttaagcgcgagactttctaagtcccggcgtctggagaatctgatcgcccagttaccaggggaaaagaaaaatggtctgtttggtaatctgattgccctcagtctggggcttaccccgaacttcaaatccaattttgacctggctgaggacgcaaagctgcagctgagcaaagatacttatgatgatgacctcgacaatctgctcgcccagattggtgaccaatatgcggatctgtttctggcagcgaagaatctttcggatgctatcttgctgtcggatattctgcgtgttaataccgaaatcaccaaagcgcctctgtctgcaagtatgatcaagagatacgacgagcaccaccaggacctgactcttcttaaggcactggtacgccaacagcttccggagaaatacaaagaaatattcttcgaccagtccaagaatggttacgcgggctacatcgatggtggtgcatcacaggaagagttctataaatttattaaaccaatccttgagaaaatggatggcacggaagagttacttgttaaacttaaccgcgaagacttgcttagaaagcaacgtacattcgacaacggctccatcccacaccagattcatttaggtgaacttcacgccatcttgcgcagacaagaagatttctatcccttcttaaaagacaatcgggagaaaatcgagaagatcctgacgttccgcattccctattatgtcggtcccctggcacgtggtaattctcggtttgcctggatgacgcgcaaaagtgaggaaaccatcaccccttggaactttgaagaagtcgtggataaaggtgctagcgcgcagtcttttatagaaagaatgacgaacttcgataaaaacttgcccaacgaaaaagtcctgcccaagcactctcttttatatgagtactttactgtgtacaacgaactgactaaagtgaaatacgttacggaaggtatgcgcaaacctgcctttcttagtggcgagcagaaaaaagcaattgtcgatcttctctttaaaacgaatcgcaaggtaactgtaaaacagctgaaggaagattatttcaaaaagatcgaatgctttgattctgtcgagatctcgggtgtcgaagatcgtttcaacgcttccttagggacctatcatgatttgctgaagataataaaagacaaagactttctcgacaatgaagaaaatgaagatattctggaggatattgttttgaccttgaccttattcgaagatagagagatgatcgaggagcgcttaaaaacctatgcccacctgtttgatgacaaagtcatgaagcaattaaagcgccgcagatatacggggtggggccgcttgagccgcaagttgattaacggtattagagacaagcagagcggaaaaactatcctggatttcctcaaatctgacggatttgcgaaccgcaattttatgcagcttatacatgatgattcgcttacattcaaagaggatattcagaaggctcaggtgtctgggcaaggtgattcactccacgaacatatagcaaatttggccggctctcctgcgattaagaaggggatcctgcaaacagttaaagttgtggatgaacttgtaaaagtaatgggccgccacaagccggagaatatcgtgatagaaatggcgcgcgagaatcaaacgacacaaaaaggtcaaaagaactcaagagagagaatgaagcgcattgaggaggggataaaggaacttggatctcaaattctgaaagaacatccagttgaaaacactcagctgcaaaatgaaaaattgtacctgtactacctgcagaatggaagagacatgtacgtggatcaggaattggatatcaatagactctcggactatgacgtagatcacattgtccctcagagcttcctcaaggatgattctatagataataaagtacttacgagatcggacaaaaatcgcggtaaatcggataacgtcccatcggaggaagtcgttaaaaagatgaaaaactattggcgtcaactgctgaacgccaagctgatcacacagcgtaagtttgataatctgactaaagccgaacgcggtggtcttagtgaactcgataaagcaggatttataaaacggcagttagtagaaacgcgccaaattacgaaacacgtggctcagatcctcgattctagaatgaatacaaagtacgatgaaaacgataaactgatccgtgaagtaaaagtcattaccttaaaatctaaacttgtgtccgatttccgcaaagattttcagttttacaaggtccgggaaatcaataactatcaccatgcacatgatgcatatttaaatgcggttgtaggcacggcccttattaagaaataccctaaactcgaaagtgagtttgtttatggggattataaagtgtatgacgttcgcaaaatgatcgcgaaatcagaacaggaaatcggtaaggctaccgctaaatactttttttattccaacattatgaatttttttaagaccgaaataactctcgcgaatggtgaaatccgtaaacggcctcttatagaaaccaatggtgaaacgggagaaatcgtttgggataaaggtcgtgactttgccaccgttcgtaaagtcctctcaatgccgcaagttaacattgtcaagaagacggaagttcaaacagggggattctccaaagaatctatcctgccgaagcgtaacagtgataaacttattgccagaaaaaaagattgggatccaaaaaaatacggaggctttgattcccctaccgtcgcgtatagtgtgctggtggttgctaaagtcgagaaagggaaaagcaagaaattgaaatcagttaaagaactgctgggtattacaattatggaaagatcgtcctttgagaaaaatccgatcgactttttagaggccaaggggtataaggaagtgaaaaaagatctcatcatcaaattaccgaagtatagtctttttgagctggaaaacggcagaaaaagaatgctggcctccgcgggcgagttacagaagggaaatgagctggcgctgccttccaaatatgttaattttctgtaccttgccagtcattatgagaaactgaagggcagccccgaagataacgaacagaaacaattattcgtggaacagcataagcactatttagatgaaattatagagcaaattagtgaattttctaagcgcgttatcctcgcggatgctaatttagacaaagtactgtcagcttataataaacatcgggataagccgattagagaacaggccgaaaatatcattcatttgtttaccttaaccaaccttggagcaccagctgccttcaaatatttcgataccacaattgatcgtaaacggtatacaagtacaaaagaagtcttggacgcaaccctcattcatcaatctattactggattatatgagacacgcattgatctttcacagctgggcggagac

SEQ ID NO: 16 - DNA, 21 bp, Trichoderma reesei
aagaagaaaaaactgaaactg

SEQ ID NO: 17 - DNA, 4284 bp, Artificial sequence
  synthetic construct
atgcaccatcatcatcatcattcttctggtctggtgccacgcggttctggtatgaaagaaaccgctgctgctaaattcgaacgccagcacatggacagcccagatctgggtaccgacgacgacgacaaggccatggccccaaaaaagaaacgcaaggttatggataaaaaatacagcattggtctggatatcggaaccaacagcgttgggtgggcagtaataacagatgaatacaaagtgccgtcaaaaaaatttaaggttctggggaatacagatcgccacagcataaaaaagaatctgattggggcattgctgtttgattcgggtgagacagctgaggccacgcgtctgaaacgtacagcaagaagacgttacacacgtcgtaaaaatcgtatttgctacttacaggaaattttttctaacgaaatggccaaggtagatgatagtttcttccatcgtctcgaagaatcttttctggttgaggaagataaaaaacacgaacgtcaccctatctttggcaatatcgtggatgaagtggcctatcatgaaaaataccctacgatttatcatcttcgcaagaagttggttgatagtacggacaaagcggatctgcgtttaatctatcttgcgttagcgcacatgatcaaatttcgtggtcatttcttaattgaaggtgatctgaatcctgataactctgatgtggacaaattgtttatacaattagtgcaaacctataatcagctgttcgaggaaaaccccattaatgcctctggagttgatgccaaagcgattttaagcgcgagactttctaagtcccggcgtctggagaatctgatcgcccagttaccaggggaaaagaaaaatggtctgtttggtaatctgattgccctcagtctggggcttaccccgaacttcaaatccaattttgacctggctgaggacgcaaagctgcagctgagcaaagatacttatgatgatgacctcgacaatctgctcgcccagattggtgaccaatatgcggatctgtttctggcagcgaagaatctttcggatgctatcttgctgtcggatattctgcgtgttaataccgaaatcaccaaagcgcctctgtctgcaagtatgatcaagagatacgacgagcaccaccaggacctgactcttcttaaggcactggtacgccaacagcttccggagaaatacaaagaaatattcttcgaccagtccaagaatggttacgcgggctacatcgatggtggtgcatcacaggaagagttctataaatttattaaaccaatccttgagaaaatggatggcacggaagagttacttgttaaacttaaccgcgaagacttgcttagaaagcaacgtacattcgacaacggctccatcccacaccagattcatttaggtgaacttcacgccatcttgcgcagacaagaagatttctatcccttcttaaaagacaatcgggagaaaatcgagaagatcctgacgttccgcattccctattatgtcggtcccctggcacgtggtaattctcggtttgcctggatgacgcgcaaaagtgaggaaaccatcaccccttggaactttgaagaagtcgtggataaaggtgctagcgcgcagtcttttatagaaagaatgacgaacttcgataaaaacttgcccaacgaaaaagtcctgcccaagcactctcttttatatgagtactttactgtgtacaacgaactgactaaagtgaaatacgttacggaaggtatgcgcaaacctgcctttcttagtggcgagcagaaaaaagcaattgtcgatcttctctttaaaacgaatcgcaaggtaactgtaaaacagctgaaggaagattatttcaaaaagatcgaatgctttgattctgtcgagatctcgggtgtcgaagatcgtttcaacgcttccttagggacctatcatgatttgctgaagataataaaagacaaagactttctcgacaatgaagaaaatgaagatattctggaggatattgttttgaccttgaccttattcgaagatagagagatgatcgaggagcgcttaaaaacctatgcccacctgtttgatgacaaagtcatgaagcaattaaagcgccgcagatatacggggtggggccgcttgagccgcaagttgattaacggtattagagacaagcagagcggaaaaactatcctggatttcctcaaatctgacggatttgcgaaccgcaattttatgcagcttatacatgatgattcgcttacattcaaagaggatattcagaaggctcaggtgtctgggcaaggtgattcactccacgaacatatagcaaatttggccggctctcctgcgattaagaaggggatcctgcaaacagttaaagttgtggatgaacttgtaaaagtaatgggccgccacaagccggagaatatcgtgatagaaatggcgcgcgagaatcaaacgacacaaaaaggtcaaaagaactcaagagagagaatgaagcgcattgaggaggggataaaggaacttggatctcaaattctgaaagaacatccagttgaaaacactcagctgcaaaatgaaaaattgtacctgtactacctgcagaatggaagagacatgtacgtggatcaggaattggatatcaatagactctcggactatgacgtagatcacattgtccctcagagcttcctcaaggatgattctatagataataaagtacttacgagatcggacaaaaatcgcggtaaatcggataacgtcccatcggaggaagtcgttaaaaagatgaaaaactattggcgtcaactgctgaacgccaagctgatcacacagcgtaagtttgataatctgactaaagccgaacgcggtggtcttagtgaactcgataaagcaggatttataaaacggcagttagtagaaacgcgccaaattacgaaacacgtggctcagatcctcgattctagaatgaatacaaagtacgatgaaaacgataaactgatccgtgaagtaaaagtcattaccttaaaatctaaacttgtgtccgatttccgcaaagattttcagttttacaaggtccgggaaatcaataactatcaccatgcacatgatgcatatttaaatgcggttgtaggcacggcccttattaagaaataccctaaactcgaaagtgagtttgtttatggggattataaagtgtatgacgttcgcaaaatgatcgcgaaatcagaacaggaaatcggtaaggctaccgctaaatactttttttattccaacattatgaatttttttaagaccgaaataactctcgcgaatggtgaaatccgtaaacggcctcttatagaaaccaatggtgaaacgggagaaatcgtttgggataaaggtcgtgactttgccaccgttcgtaaagtcctctcaatgccgcaagttaacattgtcaagaagacggaagttcaaacagggggattctccaaagaatctatcctgccgaagcgtaacagtgataaacttattgccagaaaaaaagattgggatccaaaaaaatacggaggctttgattcccctaccgtcgcgtatagtgtgctggtggttgctaaagtcgagaaagggaaaagcaagaaattgaaatcagttaaagaactgctgggtattacaattatggaaagatcgtcctttgagaaaaatccgatcgactttttagaggccaaggggtataaggaagtgaaaaaagatctcatcatcaaattaccgaagtatagtctttttgagctggaaaacggcagaaaaagaatgctggcctccgcgggcgagttacagaagggaaatgagctggcgctgccttccaaatatgttaattttctgtaccttgccagtcattatgagaaactgaagggcagccccgaagataacgaacagaaacaattattcgtggaacagcataagcactatttagatgaaattatagagcaaattagtgaattttctaagcgcgttatcctcgcggatgctaatttagacaaagtactgtcagcttataataaacatcgggataagccgattagagaacaggccgaaaatatcattcatttgtttaccttaaccaaccttggagcaccagctgccttcaaatatttcgataccacaattgatcgtaaacggtatacaagtacaaaagaagtcttggacgcaaccctcattcatcaatctattactggattatatgagacacgcattgatctttcacagctgggcggagacaagaagaaaaaactgaaactg

SEQ ID NO: 18 - protein, 46 aa, Artificial sequence
  synthetic construct
MHHHHHHSSGLVPRGSGMKETAAAKFERQHMDSPDLGTDDDDKAMA

SEQ ID NO: 19 - protein, 7 aa, SV40
PKKKRKV

SEQ ID NO: 20 - protein, 7 aa, Trichoderma reesei
KKKKLKL

SEQ ID NO: 21 - protein, 1428 aa, Artificial sequence
  protein expressed from synthetic construct
MHHHHHHSSGLVPRGSGMKETAAAKFERQHMDSPDLGTDDDDKAMAPKKKRKVMDKKYSIGLDIGTNSVGWAVITDEYKVPSKKFKVLGNTDRHSIKKNLIGALLFDSGETAEATRLKRTARRRYTRRKNRICYLQEIFSNEMAKVDDSFFHRLEESFLVEEDKKHERHPIFGNIVDEVAYHEKYPTIYHLRKKLVDSTDKADLRLIYLALAHMIKFRGHFLIEGDLNPDNSDVDKLFIQLVQTYNQLFEENPINASGVDAKAILSARLSKSRRLENLIAQLPGEKKNGLFGNLIALSLGLTPNFKSNFDLAEDAKLQLSKDTYDDDLDNLLAQIGDQYADLFLAAKNLSDAILLSDILRVNTEITKAPLSASMIKRYDEHHQDLTLLKALVRQQLPEKYKEIFFDQSKNGYAGYIDGGASQEEFYKFIKPILEKMDGTEELLVKLNREDLLRKQRTFDNGSIPHQIHLGELHAILRRQEDFYPFLKDNREKIEKILTFRIPYYVGPLARGNSRFAWMTRKSEETITPWNFEEVVDKGASAQSFIERMTNFDKNLPNEKVLPKHSLLYEYFTVYNELTKVKYVTEGMRKPAFLSGEQKKAIVDLLFKTNRKVTVKQLKEDYFKKIECFDSVEISGVEDRFNASLGTYHDLLKIIKDKDFLDNEENEDILEDIVLTLTLFEDREMIEERLKTYAHLFDDKVMKQLKRRRYTGWGRLSRKLINGIRDKQSGKTILDFLKSDGFANRNFMQLIHDDSLTFKEDIQKAQVSGQGDSLHEHIANLAGSPAIKKGILQTVKVVDELVKVMGRHKPENIVIEMARENQTTQKGQKNSRERMKRIEEGIKELGSQILKEHPVENTQLQNEKLYLYYLQNGRDMYVDQELDINRLSDYDVDHIVPQSFLKDDSIDNKVLTRSDKNRGKSDNVPSEEVVKKMKNYWRQLLNAKLITQRKFDNLTKAERGGLSELDKAGFIKRQLVETRQITKHVAQILDSRMNTKYDENDKLIREVKVITLKSKLVSDFRKDFQFYKVREINNYHHAHDAYLNAVVGTALIKKYPKLESEFVYGDYKVYDVRKMIAKSEQEIGKATAKYFFYSNIMNFFKTEITLANGEIRKRPLIETNGETGEIVWDKGRDFATVRKVLSMPQVNIVKKTEVQTGGFSKESILPKRNSDKLIARKKDWDPKKYGGFDSPTVAYSVLVVAKVEKGKSKKLKSVKELLGITIMERSSFEKNPIDFLEAKGYKEVKKDLIIKLPKYSLFELENGRKRMLASAGELQKGNELALPSKYVNFLYLASHYEKLKGSPEDNEQKQLFVEQHKHYLDEIIEQISEFSKRVILADANLDKVLSAYNKHRDKPIREQAENIIHLFTLTNLGAPAAFKYFDTTIDRKRYTSTKEVLDATLIHQSITGLYETRIDLSQLGGDKKKKLKL

SEQ ID NO: 22 - DNA, 842 bp, Trichoderma reesei
aaaaaacactagtaagtacttacttatgtattattaactactttagctaacttctgcagtactacctaagaggctaggggtagttttatagcagacttatagctattatttttatttagtaaagtgcttttaaagtaaggtcttttttatagcactttttatttattataatatatattatataataattttaagcctggaatagtaaagaggcttatataataatttatagtaataaaagcttagcagctgtaatataattcctaaagaaacagcatgaaatggtattatgtaagagctatagtctaaaggcactctgctggataaaaatagtggctataagtctgctgcaaaactacccccaacctcgtaggtatataagtactgtttgatggtagtctatcgccttcgggcatttggtcaatttataacgatacaggttcgtttcggcttttcctcggaacccccagaggtcatcagttcgaatcgctaacaggtcaacagagaagattagcatggcccctgcactaaggatgacacgctcactcaaagagaagctaaacattttttttctcttccaagtcgtgatggttatctttttgcttagagaatctattcttgtggacgattagtattggtaaatccctgctgcacattgcggcggatggtctcaacggcataataccccattcgtgatgcagcggtgatcttcaatatgtagtgtaatacgttgcatacaccaccaggttcggtgcctcctgtatgtacagtactgtagttcgactcctccgcgcaggtggaaacgattccctagtgggcaggtattttggcggggtcaagaa

SEQ ID NO: 23 - RNA, 99 nt, Artificial sequence
  sg RNA
  misc_feature (1)..(20): N region - complementary to target site
nnnnnnnnnnnnnnnnnnnnguuuuagagcuagaaauagcaaguuaaaauaaggcuaguccguuaucaacuugaaaaaguggcaccgagucgguggugc

SEQ ID NO: 24 - RNA, 99 nt, Artificial sequence
  Synthetic construct
guccucgagcaaaaggugccguuuuagagcuagaaauagcaaguuaaaauaaggcuaguccguuaucaacuugaaaaaguggcaccgagucgguggugc

SEQ ID NO: 25 - RNA, 99 nt, Artificial sequence
  Synthetic construct
guucagugcaauaggcgucuguuuuagagcuagaaauagcaaguuaaaauaaggcuaguccguuaucaacuugaaaaaguggcaccgagucgguggugc

SEQ ID NO: 26 - RNA, 99 nt, Artificial sequence
  Synthetic construct
gccaauggcgacggcagcacguuuuagagcuagaaauagcaaguuaaaauaaggcuaguccguuaucaacuugaaaaaguggcaccgagucgguggugc

SEQ ID NO: 27 - RNA, 99 nt, Artificial sequence
  Synthetic construct
gcacagcgggaugcccuuguguuuuagagcuagaaauagcaaguuaaaauaaggcuaguccguuaucaacuugaaaaaguggcaccgagucgguggugc

SEQ ID NO: 28 - DNA, 412 bp, Artificial sequence
  Synthetic construct
gaattcggatcctctttgaaaagataatgtatgattatgctttcactcatatttatacagaaacttgatgttttctttcgagtatatacaaggtgattacatgtacgtttgaagtacaactctagattttgtagtgccctcttgggctagcggtaaaggtgcgcattttttcacaccctacaatgttctgttcaaaagattttggtcaaacgctgtagaagtgaaagttggtgcgcatgtttcggcgttcgaaacttctccgcagtgaaagataaatgatcgtcctcgagcaaaaggtgccgttttagagctagaaatagcaagttaaaataaggctagtccgttatcaacttgaaaaagtggcaccgagtcggtggtgctttttttgttttttatgtctgaattcggatcc

SEQ ID NO: 29 - DNA, 540 bp, Artificial sequence
  Synthetic construct
gaattcggatccaaaaaacactagtaagtacttacttatgtattattaactactttagctaacttctgcagtactacctaagaggctaggggtagttttatagcagacttatagctattatttttatttagtaaagtgcttttaaagtaaggtcttttttatagcactttttatttattataatatatattatataataattttaagcctggaatagtaaagaggcttatataataatttatagtaataaaagcttagcagctgtaatataattcctaaagaaacagcatgaaatggtattatgtaagagctatagtctaaaggcactctgctggataaaaatagtggctataagtctgctgcaaaactacccccaacctcgtaggtatataagtactgtttgatggtagtctatcgtcctcgagcaaaaggtgccgttttagagctagaaatagcaagttaaaataaggctagtccgttatcaacttgaaaaagtggcaccgagtcggtggtgcttttttttctcttgaattcggatcc

SEQ ID NO: 30 - DNA, 597 bp, Artificial sequence
  Synthetic construct
gaattcggatccaaaaaacactagtaagtacttacttatgtattattaactactttagctaacttctgcagtactacctaagaggctaggggtagttttatagcagacttatagctattatttttatttagtaaagtgcttttaaagtaaggtcttttttatagcactttttatttattataatatatattatataataattttaagcctggaatagtaaagaggcttatataataatttatagtaataaaagcttagcagctgtaatataattcctaaagaaacagcatgaaatggtattatgtaagagctatagtctaaaggcactctgctggataaaaatagtggctataagtctgctgcaaaactacccccaacctcgtaggtatataagtactgtttgatggtagtctatcgtcctcgagcaaaaggtgccgttttagagctagagttcgtttcggcttttcctcggaacccccagaggtcatcagttcgaatcgctaacagaatagcaagttaaaataaggctagtccgttatcaacttgaaaaagtggcaccgagtcggtggtgcttttttttctcttgaattcggatcc

SEQ ID NO: 31 - DNA, 315 bp, Artificial sequence
  Synthetic construct
aattcctaaagaaacagcatgaaatggtattatgtaagagctatagtctaaaggcactctgctggataaaaatagtggctataagtctgctgcaaaactacccccaacctcgtaggtatataagtactgtttgatggtagtctatcgccaatggcgacggcagcacgttttagagctagagttcgtttcggcttttcctcggaacccccagaggtcatcagttcgaatcgctaacagaatagcaagttaaaataaggctagtccgttatcaacttgaaaaagtggcaccgagtcggtggtgcttttttttctctt

SEQ ID NO: 32 - DNA, 39 bp, Artificial sequence
  primer
cgtcagcttaagaattcctaaagaaacagcatgaaatgg

SEQ ID NO: 33 - DNA, 47 bp, Artificial sequence
  primer
cgtcagggccacgtgggccaagagaaaaaaaagcaccaccgactcgg

SEQ ID NO: 34 - DNA, 23 bp, Artificial sequence
  primer
tgaacacagccaccgacatcagc

SEQ ID NO: 35 - DNA, 23 bp, Artificial sequence
  primer
gctggtgagggtttgtgctattg

SEQ ID NO: 36 - DNA, 21 bp, Artificial sequence
  primer
gattgcttgggaggaggacat

SEQ ID NO: 37 - DNA, 23 bp, Artificial sequence
  primer
cgaggccactgatgaagttgttc

SEQ ID NO: 38 - DNA, 23 bp, Artificial sequence
  primer
cagttttccaaggctgccaacgc

SEQ ID NO: 39 - DNA, 22 bp, Artificial sequence
  primer
ctgatcttgcaccctggaaatc

SEQ ID NO: 40 - DNA, 23 bp, Artificial sequence
  primer
ctctctatcatttgccaccctcc

SEQ ID NO: 41 - DNA, 22 bp, Artificial sequence
  primer
ctccattcaccctcaattctcc

SEQ ID NO: 42 - DNA, 23 bp, Artificial sequence
  primer
gttcccttggcggtgcttggatc

SEQ ID NO: 43 - DNA, 23 bp, Artificial sequence
  primer
caatagcacaaaccctcaccagc

SEQ ID NO: 44 - DNA, 23 bp, Artificial sequence
  primer
gaacaacttcatcagtggcctcg

SEQ ID NO: 45 - DNA, 23 bp, Artificial sequence
  primer
ccgttagttgaagatccttgccg

SEQ ID NO: 46 - DNA, 23 bp, Artificial sequence
  primer
gtcgaggatttgcttcatacctc

SEQ ID NO: 47 - DNA, 23 bp, Artificial sequence
  primer
tgccgactttgtccagtgattcg

SEQ ID NO: 48 - DNA, 23 bp, Artificial sequence
  primer
ttacatgtggacgcgagatagcg

SEQ ID NO: 49 - DNA, 22 bp, Artificial sequence
  primer
gtgtgtctaatgcctccaccac

SEQ ID NO: 50 - DNA, 22 bp, Artificial sequence
  primer
gatcgtgctagcgctgctgttg

SEQ ID NO: 51 - DNA, 21 bp, Artificial sequence
  primer
ccgtgatggagcccgtcttct

SEQ ID NO: 52 - DNA, 22 bp, Artificial sequence
  primer
cgcggtgagttcaggctttttc

SEQ ID NO: 53 - DNA, 22 bp, Artificial sequence
  primer
gtataagagcaggaggagggag

SEQ ID NO: 54 - DNA, 22 bp, Artificial sequence
  primer
gaacgcctcaatcagtcagtcg

SEQ ID NO: 55 - DNA, 2431 bp, Artificial sequence
  Synthetic construct
tcaggaaatagctttaagtagcttattaagtattaaaattatatatatttttaatataactatatttctttaataaataggtattttaagctttatatataaatataataataaaataatatattatatagctttttattaataaataaaatagctaaaaatataaaaaaaatagctttaaaatacttatttttaattagaattttatatatttttaatatataagatcttttacttttttataagcttcctaccttaaattaaatttttacttttttttactattttactatatcttaaataaaggctttaaaaatataaaaaaaatcttcttatatattataagctataaggattatatatatatttttttttaatttttaaagtaagtattaaagctagaattaaagttttaattttttaaggctttatttaaaaaaaggcagtaatagcttataaaagaaatttctttttcttttatactaaaagtactttttttttaataaggttagggttagggtttactcacaccgaccatcccaaccacatcttagggttagggttagggttagggttagggttagggttagggttagggtaagggtttaaacaaagccacgttgtgtctcaaaatctctgatgttacattgcacaagataaaaatatatcatcatgaacaataaaactgtctgcttacataaacagtaatacaaggggtgttatgagccatattcaacgggaaacgtcttgctcgaggccgcgattaaattccaacatggatgctgatttatatgggtataaatgggctcgcgataatgtcgggcaatcaggtgcgacaatctatcgattgtatgggaagcccgatgcgccagagttgtttctgaaacatggcaaaggtagcgttgccaatgatgttacagatgagatggtcagactaaactggctgacggaatttatgcctcttccgaccatcaagcattttatccgtactcctgatgatgcatggttactcaccactgcgatccccgggaaaacagcattccaggtattagaagaatatcctgattcaggtgaaaatattgttgatgcgctggcagtgttcctgcgccggttgcattcgattcctgtttgtaattgtccttttaacagcgatcgcgtatttcgtctcgctcaggcgcaatcacgaatgaataacggtttggttgatgcgagtgattttgatgacgagcgtaatggctggcctgttgaacaagtctggaaagaaatgcataagcttttgccattctcaccggattcagtcgtcactcatggtgatttctcacttgataaccttatttttgacgaggggaaattaataggttgtattgatgttggacgagtcggaatcgcagaccgataccaggatcttgccatcctatggaactgcctcggtgagttttctccttcattacagaaacggctttttcaaaaatatggtattgataatcctgatatgaataaattgcagtttcatttgatgctcgatgagtttttctaatcagaattggttaattggttgtaacactggcagagcattacgctgacttgacgggacggcggctttgttgaataaatcgaacttttgctgagttgaaggatcagatcacgcatcttcccgacaacgcagaccgttccgtggcaaagcaaaagttcaaaatcaccaactggtccacctacaacaaagctctcatcaaccgtggctccctcactttctggctggatgatggggcgattcaggcctggtatgagtcagcaacaccttcttcacgaggcagacctcagcggtttaaacctaaccctaaccctaaccctaaccctaaccctaaccctaaccctaaccctaaccctaaccctaaccctaaccctaaccctaacctaaccctaatggggtcgatctgaaccgaggatgagggttctatagactaatctacaggccgtacatggtgtgattgcagatgcgacgggcaaggtgtacagtgtccagaaggaggagagcggcataggtattgtaatagaccagctttacataataatcgcctgttgctactgactgatgaccttcttccctaaccagtttcctaattaccactgcagtgaggataaccctaactcgctctggggttattattatactgattagcaggtggcttatatagtgctgaagtactataagagtttctgcgggaggaggtggaaggactataaactggacacagttagggatagagtgatgacaagacctgaatgttatcctccggtgtggtatagcgaattggctgaccttgcagatggtaatggtttaggcagggtttttgcagagggggacgagaacgcgttctgcgatttaacggctgctgccgccaagctttacggttctctaatgggcggccgc

SEQ ID NO: 56 - DNA, 23 bp, Trichoderma reesei
gcagcacctcgcacagcatgcgg

SEQ ID NO: 57 - DNA, 23 bp, Artificial sequence
  linker
taggcagcacctcgcacagcatg

SEQ ID NO: 58 - DNA, 22 bp, Artificial sequence
  linker
aaaccatgctgtgcgaggtgct

SEQ ID NO: 59 - DNA, 23 bp, Trichoderma reesei
gctgccaggaagaattcaacggg

SEQ ID NO: 60 - DNA, 23 bp, Artificial sequence
  linker
taggctgccaggaagaattcaac

SEQ ID NO: 61 - DNA, 22 bp, Artificial sequence
  linker
aaacgttgaattcttcctggca

SEQ ID NO: 62 - DNA, 23 bp, Trichoderma reesei
gctcaagacgcactacgacatgg

SEQ ID NO: 63 - DNA, 23 bp, Artificial sequence
  linker
taggctcaagacgcactacgaca

SEQ ID NO: 64 - DNA, 24 bp, Artificial sequence
  linker
aaactgtcgtagtgcgtcttgagc

SEQ ID NO: 65 - DNA, 123 bp, Artificial sequence
  Synthetic construct
taatacgactcactatagggcagcacctcgcacagcatggttttagagctagaaatagcaagttaaaataaggctagtccgttatcaacttgaaaaagtggcaccgagtcggtgctttttacg

SEQ ID NO: 66 - DNA, 123 bp, Artificial sequence
  Synthetic construct
taatacgactcactatagggctgccaggaagaattcaacgttttagagctagaaatagcaagttaaaataaggctagtccgttatcaacttgaaaaagtggcaccgagtcggtgctttttacg

SEQ ID NO: 67 - DNA, 123 bp, Artificial sequence
  Synthetic construct
taatacgactcactatagggctcaagacgcactacgacagttttagagctagaaatagcaagttaaaataaggctagtccgttatcaacttgaaaaagtggcaccgagtcggtgctttttacg

SEQ ID NO: 68 - DNA, 47 bp, Trichoderma reesei
tggcccgtcgattgtcgtgctcaagacgcactacgacatggtctcgg

SEQ ID NO: 69 - DNA, 49 bp, unknown
  mutant T4 4-3
tggcccgtcgattgtcgtgctcaagacgcactacgcgacatggtctcgg

SEQ ID NO: 70 - DNA, 47 bp, unknown; identical to SEQ ID NO: 68
  mutant T4 4-13

SEQ ID NO: 71 - DNA, 48 bp, unknown
  mutant T4 4-11
tggcccgtcgattgtcgtgctcaagacgcactacggacatggtctcgg

SEQ ID NO: 72 - DNA, 47 bp, unknown; identical to SEQ ID NO: 68
  mutant T4 4-12

SEQ ID NO: 73 - DNA, 48 bp, unknown; identical to SEQ ID NO: 71
  mutant T4 4-18

SEQ ID NO: 74 - DNA, 115 bp, unknown
  mutant T4 4-20
tggcccgtcgattgtcgtgctcaagacgcactacgagccgacagggcgcctggctaaatccaaggtcaagacaggctggtggttgtttagtgcgagtcctctgacatggtctcgg

SEQ ID NO: 75 - DNA, 48 bp, unknown; identical to SEQ ID NO: 71
  mutant T4 4-19

SEQ ID NO: 76 - DNA, 48 bp, unknown
  mutant T4 4-4
tggcccgtcgaatgttgtggtcaaggcgcccttcggacatggtctcgg

SEQ ID NO: 77 - DNA, 48 bp, unknown; identical to SEQ ID NO: 71
  mutant T4 4-7

SEQ ID NO: 78 - DNA, 187 bp, unknown
  mutant T4 2.2
ccgctgacggcttacctgttcaagctcatggacctcaaggcgtccaacctgtgcctgagcgccgacgtgccgacagcgcgcgagctgctgtacctggccgacaagattggcccgtcgattgtcgtgctcaagacgcactacgcaggcctgcgtcgaggccgcccgggagcacaaggactttgtcatg

SEQ ID NO: 79 - DNA, 798 bp, Trichoderma reesei
ccgctgacggcttacctgttcaagctcatggacctcaaggcgtccaacctgtgcctgagcgccgacgtgccgacagcgcgcgagctgctgtacctggccgacaagattggcccgtcgattgtcgtgctcaagacgcactacgacatggtctcgggctgggacttccacccggagacgggcacgggagcccagctggcgtcgctggcgcgcaagcacggcttcctcatcttcgaggaccgcaagtttggcgacattggccacaccgtcgagctgcagtacacgggcgggtcggcgcgcatcatcgactgggcgcacattgtcaacgtcaacatggtgcccggcaaggcgtcggtggcctcgctggcccagggcgccaagcgctggctcgagcgctacccctgcgaggtcaagacgtccgtcaccgtcggcacgcccaccatggactcgtttgacgacgacgccgactccagggacgccgagcccgccggcgccgtcaacggcatgggctccattggcgtcctggacaagcccatctactcgaaccggtccggcgacggccgcaagggcagcatcgtctccatcaccaccgtcacccagcagtacgagtccgtctcctcgccccggttaacaaaggccatcgccgagggcgacgagtcgctcttcccgggcatcgaggaggcgccgctgagccgcggcctcctgatcctcgcccaaatgtccagccagggcaacttcatgaacaaggagtacacgcaggcctgcgtcgaggccgcccgggagcacaaggactttgtcatg

SEQ ID NO: 80 - DNA, 59 bp, Trichoderma reesei
ctggccgacaagattggcccgtcgattgtcgtgctcaagacgcactacgacatggtctc

SEQ ID NO: 81 - DNA, 60 bp, unknown
  mutant T4 2.4
ctggccgacaagattggcccgtcgattgtcgtgctcaagacgcactacggacatggtctc

SEQ ID NO: 82 - DNA, 101 bp, Artificial sequence
  consensus sequence
gacagcgcgcgagctgctgtacctggccgacaagattggcccgtcgattgtcgtgctcaagacgcactacgacatggtctcgggctgggacttccacccgg

SEQ ID NO: 83 - DNA, 102 bp, unknown
  mutant P37 #13 4.2
gacagcgcgcgagctgctgtacctggccgacaagattggcccgtcgattgtcgtgctcaagacgcactacggacatggtctcgggctgggacttccacccgg

SEQ ID NO: 84 - DNA, 102 bp, unknown
  mutant P37 4.1 #12
gacagcgcgcgagctgctgtacctggccgacaagattggcccgtcgattgtcgtgctcaagacgcactacgtacatggtctcgggctgggacttccacccgg

SEQ ID NO: 85 - DNA, 100 bp, unknown
  mutant P37 #15 4.4
gacagcgcgcgagctgctgtacctggccgacaagattggcccgtcgattgtcgtgctcaagacgcactacgcatggtctcgggctgggacttccacccgg

SEQ ID NO: 86 - DNA, 101 bp, unknown; identical to SEQ ID NO: 82
  mutant P37 #14 4.3

SEQ ID NO: 87 - DNA, 101 bp, Artificial sequence
  consensus sequence
  misc_feature (67)..(68): n is a, c, g, or t
  misc_feature (70)..(70): n is a, c, g, or t
  misc_feature (72)..(75): n is a, c, g, or t
  misc_feature (78)..(82): n is a, c, g, or t
  misc_feature (85)..(86): n is a, c, g, or t
  misc_feature (91)..(93): n is a, c, g, or t
  misc_feature (95)..(95): n is a, c, g, or t
  misc_feature (97)..(97): n is a, c, g, or t
  misc_feature (99)..(99): n is a, c, g, or t
gacagcgcgcgagctgctgtacctggccgacaagattggcccgtcgattgtcgtgctcaagacgcannangnnnnggnnnnnggnngggannncnancngg

SEQ ID NO: 88 - DNA, 1146 bp, Trichoderma reesei
atggcaccacacccgacgctcaaggccaccttcgcggccaggagcgagacggcgacgcacccgctgacggcttacctgttcaagctcatggacctcaaggcgtccaacctgtgcctgagcgccgacgtgccgacagcgcgcgagctgctgtacctggccgacaagattggcccgtcgattgtcgtgctcaagacgcactacgacatggtctcgggctgggacttccacccggagacgggcacgggagcccagctggcgtcgctggcgcgcaagcacggcttcctcatcttcgaggaccgcaagtttggcgacattggccacaccgtcgagctgcagtacacgggcgggtcggcgcgcatcatcgactgggcgcacattgtcaacgtcaacatggtgcccggcaaggcgtcggtggcctcgctggcccagggcgccaagcgctggctcgagcgctacccctgcgaggtcaagacgtccgtcaccgtcggcacgcccaccatggactcgtttgacgacgacgccgactccagggacgccgagcccgccggcgccgtcaacggcatgggctccattggcgtcctggacaagcccatctactcgaaccggtccggcgacggccgcaagggcagcatcgtctccatcaccaccgtcacccagcagtacgagtccgtctcctcgccccggttaacaaaggccatcgccgagggcgacgagtcgctcttcccgggcatcgaggaggcgccgctgagccgcggcctcctgatcctcgcccaaatgtccagccagggcaacttcatgaacaaggagtacacgcaggcctgcgtcgaggccgcccgggagcacaaggactttgtcatgggcttcatctcgcaggagacgctcaacaccgagcccgacgatgcctttatccacatgacgcccggctgccagctgccccccgaagacgaggaccagcagaccaacggatcggtcggtggagacggccagggccagcagtacaacacgccgcacaagctgattggcatcgccggcagcgacattgccattgtgggccggggcatcctcaaggcctcagaccccgtagaggaggcagagcggtaccgatcagcagcgtggaaagcctacaccgagaggctgctgcgatag

SEQ ID NO: 89 - DNA, 2950 bp, Trichoderma reesei
atgttgtccaatcctctccgtcgctattctgcctaccccgacatctcctcggcgtcatttgacccgaactaccatggctcacagtcgcatctccactcgatcaacgtcaacacattcggcaacagccacccctatcccatgcagcacctcgcacagcatgcggagctttcgagttcacgcatgataagggccagtccggtgcagccaaagcagcgccagggctctcttattgctgccaggaagaattcaacgggtactgctgggcccattcggcggaggatcagtcgcgcttgtgaccagtgcaaccagcttcgtaccaagtgcgatggcttacacccatgtgcccattgtataggtatgtcccttttcctctacacagtgatgctgcgctcaagcacatgtactgatcgatcttgtttagaattcggccttggatgcgaatatgtccgagagagaaagaagcgtggcaaagcttcgcgcaaggatattgctgcccagcaagccgcggcggctgcagcacaacactccggccaggtccaggatggtccagaggatcaacatcgcaaactctcacgccagcaaagcgaatcttcgcgtggcagcgctgagcttgcccagcctgcccacgacccgcctcatggccacattgagggctctgtcagctccttcagcgacaatggcctttcccagcatgctgccatgggcggcatggatggcctggaagatcaccatggccacgtcggagttgatcctgccctgggccgaactcagctggaagcgtcatcagcaatgggcctgggcgcatacggtgaagtccaccccggctatgagagccccggcatgaatggccatgtgatggtgcccccgtcgtatggcgcgcagaccaccatggccgggtattccggtatctcgtatgctgcgcaagccccgagtccggctacgtatagcagcgacggtaactttcgactcaccggtcacatccatgattacccgctggcaaatgggagctcgccctcatggggagtctcgctggcctcgccttcgaaccagttccagcttcagctctcgcagcccatcttcaagcaaagcgatttgcgatatcctgtgcttgagcctctgctgcctcacctgggaaacatcctccccgtgtctttggcgtgcgatctgattgacctgtacttctcctcgtcttcatcagcacagatgcacccaatgtccccatacgttctgggcttcgtcttccggaagcgctccttcttgcaccccacgaacccacgaaggtgccagcccgcgctgcttgcgagcatgctgtgggtggcggcacagactagcgaagcgtccttcttgacgagcctgccgtcggcgaggagcaaggtctgccagaagctgctcgagctgaccgttgggcttcttcagcccctgatccacaccggcaccaacagcccgtctcccaagactagccccgtcgtcggtgctgctgccctgggagttcttggggtggccatgccgggctcgctgaacatggattcactggccggcgaaacgggtgcttttggggccatagggagccttgacgacgtcatcacctatgtgcacctcgccacggtcgtctcggccagcgagtacaagggcgccagcctgcggtggtggggtgcggcatggtctctcgccagagagctcaagcttggccgtgagctgccgcctggcaatccacctgccaaccaggaggacggcgagggccttagcgaagacgtggatgagcacgacttgaacagaaacaacactcgcttcgtgacggaagaggagcgcgaagagcgacggcgagcatggtggctcgtttacatcgtcgacaggcacctggcgctctgctacaaccgccccttgtttcttctggacagcgagtgcagcgacttgtaccacccgatggacgacatcaagtggcaggcaggcaaatttcgcagccacgatgcagggaactccagcatcaacatcgatagctccatgacggacgagtttggcgatagtccccgggcggctcgcggcgcacactacgagtgccgcggtcgtagcatttttggctacttcttgtccttgatgacaatcctgggcgagattgtcgatgtccaccatgctaaaagccacccccggttcggcgttggattccgctccgcgcgggattgggacgagcaggttgctgaaatcacccgacacctggacatgtatgaggagagcctcaagaggttcgtggccaagcatctgccattgtcctcaaaggacaaggagcagcatgagatgcacgacagtggagcggtaacagacatgcaatctccactctcggtgcggaccaacgcgtccagccgcatgacggagagcgagatccaggccagcatcgtggtggcttacagcacccatgtgatgcatgtcctccacatcctccttgcggataagtgggatcccatcaaccttctagacgacgacgacttgtggatctcgtcggaaggattcgtgacggcgacgagccacgcggtatcggctgccgaagctattagccagattctcgagtttgaccctggcctggagtttatgccattcttctacggcgtctatctcctgcagggttccttcctcctcctgctcatcgccgacaagctgcaggccgaagcgtctccaagcgtcatcaaggcttgcgagaccattgttagggcacacgaagcttgcgttgtgacgctgagcacagagtatcaggtaagccctatcagttcaaacgtctatcttgctgtgaatcaaagactgacttggacatcagcgcaactttagcaaggttatgcgaagcgcgctggctctgattcggggccgtgtgccggaagatttagctgagcagcagcagcgacgacgcgagcttcttgcactataccgatggactggtaacggaaccggtctggccctctaa

SEQ ID NO: 90 - DNA, 57 bp, Trichoderma reesei
gttcgtttcggcttttcctcggaacccccagaggtcatcagttcgaatcgctaacag

SEQ ID NO: 91 - DNA, 13 bp, Trichoderma reesei
ttttttttctctt

SEQ ID NO: 92 - DNA, 20 bp, T. Reesei
gctcaagacgcactacgaca